European Patent Application EP 4 265 728 A1, published October 25, 2023. Title: DNA CONSTRUCT, VECTOR, BACTERIA AND METHOD OF PRODUCING POLYPEPTIDES. Applicant: Denka Company Limited. The sequence listing filed with the application follows.

SEQUENCE LISTING (14 sequences)

SEQ ID NO: 1 - protein, 386 aa, Artificial Sequence
  PDE (precursor form)
MSGSRPGCHRRDHQVHRIRTELEKHVALDLPRLPRLPRLPRAALVVTGTAALLSPAAVGTAAAAESAAPSLSVMAFNVEQLPSITELAGTPGSDRRAERREAAAVVIKRENADVVVLDEAFNKYAQAMRAMELKEVYPYQTSLVGEYCSGSGRWTSYEGNCSNSPFVVNGGVTLLSKYPILESHQLVYRNSDSKTSDYKSNKGAALARLSVNGQSVWVAGTHLQADEEGSSPVGNTRKVRLEQLKELRAWASDKAGGAPVVVAGDFNVEYYTTDPKNGHAPGTGVSGEVAKANEALGGVLATPGTTGYTYDMVDNPRARLRDDKDNGYAKYRNRLDYIGYIKGTGTQPSFSDERIVGYDGLRKGGDPLAEIPSDHQPIVSRVTVGR

SEQ ID NO: 2 - protein, 320 aa, Artificial Sequence
  PDE
AAPSLSVMAFNVEQLPSITELAGTPGSDRRAERREAAAVVIKRENADVVVLDEAFNKYAQAMRAMELKEVYPYQTSLVGEYCSGSGRWTSYEGNCSNSPFVVNGGVTLLSKYPILESHQLVYRNSDSKTSDYKSNKGAALARLSVNGQSVWVAGTHLQADEEGSSPVGNTRKVRLEQLKELRAWASDKAGGAPVVVAGDFNVEYYTTDPKNGHAPGTGVSGEVAKANEALGGVLATPGTTGYTYDMVDNPRARLRDDKDNGYAKYRNRLDYIGYIKGTGTQPSFSDERIVGYDGLRKGGDPLAEIPSDHQPIVSRVTVGR

SEQ ID NO: 3 - protein, 8 aa, Artificial Sequence
  C-terminal of PDE + linker
  MISC_FEATURE (4)..(4): Xaa = Gly or Ala
VTVXRGGG

SEQ ID NO: 4 - protein, 331 aa, Artificial Sequence
  PDE-GS-His
AAPSLSVMAFNVEQLPSITELAGTPGSDRRAERREAAAVVIKRENADVVVLDEAFNKYAQAMRAMELKEVYPYQTSLVGEYCSGSGRWTSYEGNCSNSPFVVNGGVTLLSKYPILESHQLVYRNSDSKTSDYKSNKGAALARLSVNGQSVWVAGTHLQADEEGSSPVGNTRKVRLEQLKELRAWASDKAGGAPVVVAGDFNVEYYTTDPKNGHAPGTGVSGEVAKANEALGGVLATPGTTGYTYDMVDNPRARLRDDKDNGYAKYRNRLDYIGYIKGTGTQPSFSDERIVGYDGLRKGGDPLAEIPSDHQPIVSRVTVGRGGGGSHHHHHH

SEQ ID NO: 5 - protein, 328 aa, Artificial Sequence
  His-SG-PDE
HHHHHHSGAAPSLSVMAFNVEQLPSITELAGTPGSDRRAERREAAAVVIKRENADVVVLDEAFNKYAQAMRAMELKEVYPYQTSLVGEYCSGSGRWTSYEGNCSNSPFVVNGGVTLLSKYPILESHQLVYRNSDSKTSDYKSNKGAALARLSVNGQSVWVAGTHLQADEEGSSPVGNTRKVRLEQLKELRAWASDKAGGAPVVVAGDFNVEYYTTDPKNGHAPGTGVSGEVAKANEALGGVLATPGTTGYTYDMVDNPRARLRDDKDNGYAKYRNRLDYIGYIKGTGTQPSFSDERIVGYDGLRKGGDPLAEIPSDHQPIVSRVTVGR

SEQ ID NO: 6 - protein, 326 aa, Artificial Sequence
  PDE-His
AAPSLSVMAFNVEQLPSITELAGTPGSDRRAERREAAAVVIKRENADVVVLDEAFNKYAQAMRAMELKEVYPYQTSLVGEYCSGSGRWTSYEGNCSNSPFVVNGGVTLLSKYPILESHQLVYRNSDSKTSDYKSNKGAALARLSVNGQSVWVAGTHLQADEEGSSPVGNTRKVRLEQLKELRAWASDKAGGAPVVVAGDFNVEYYTTDPKNGHAPGTGVSGEVAKANEALGGVLATPGTTGYTYDMVDNPRARLRDDKDNGYAKYRNRLDYIGYIKGTGTQPSFSDERIVGYDGLRKGGDPLAEIPSDHQPIVSRVTVGRHHHHHH

SEQ ID NO: 7 - protein, 339 aa, Artificial Sequence
  His-SG-PDE-GS-His
HHHHHHSGAAPSLSVMAFNVEQLPSITELAGTPGSDRRAERREAAAVVIKRENADVVVLDEAFNKYAQAMRAMELKEVYPYQTSLVGEYCSGSGRWTSYEGNCSNSPFVVNGGVTLLSKYPILESHQLVYRNSDSKTSDYKSNKGAALARLSVNGQSVWVAGTHLQADEEGSSPVGNTRKVRLEQLKELRAWASDKAGGAPVVVAGDFNVEYYTTDPKNGHAPGTGVSGEVAKANEALGGVLATPGTTGYTYDMVDNPRARLRDDKDNGYAKYRNRLDYIGYIKGTGTQPSFSDERIVGYDGLRKGGDPLAEIPSDHQPIVSRVTVGRGGGGSHHHHHH

SEQ ID NO: 8 - protein, 334 aa, Artificial Sequence
  His-SG-PDE-His
HHHHHHSGAAPSLSVMAFNVEQLPSITELAGTPGSDRRAERREAAAVVIKRENADVVVLDEAFNKYAQAMRAMELKEVYPYQTSLVGEYCSGSGRWTSYEGNCSNSPFVVNGGVTLLSKYPILESHQLVYRNSDSKTSDYKSNKGAALARLSVNGQSVWVAGTHLQADEEGSSPVGNTRKVRLEQLKELRAWASDKAGGAPVVVAGDFNVEYYTTDPKNGHAPGTGVSGEVAKANEALGGVLATPGTTGYTYDMVDNPRARLRDDKDNGYAKYRNRLDYIGYIKGTGTQPSFSDERIVGYDGLRKGGDPLAEIPSDHQPIVSRVTVGRHHHHHH

SEQ ID NO: 9 - protein, 5 aa, Artificial Sequence
  linker
GGGGS

SEQ ID NO: 10 - protein, 7 aa, Artificial Sequence
  His Tag
MHHHHHH

SEQ ID NO: 11 - protein, 350 aa, Artificial Sequence
  PDE
MTAKTPRTALAAAGAALILSPLPTGTAVAAEKAPAISVMAFNVEQLPSITEIARTWGSDRRTERATVAAEVIRRENPDVVVLDEAFNKYAQAMRTDLRKAYPHQSSLVGEHCGGKGNWTSYAGNCSNSPIVVNGGVTVLSKYPILESHQLVYSDSDRKTSDYKSNKGAALVRLSVDGAPVWVAGTHLQADEESGSPIENTRKVRLRQLRELRSWATEKSGGRPVIVAGDLNVEYHATDPRDGRAPTGAVSADVAEADGALGGKLSPQHITQHTYDMVGNARAKLRDDAKGSYAKYRNRLDYIGYINGTGPAPTFTDGRVVSYAGLHKGGDPLAEIPSDHQPLVSRVTVAR

SEQ ID NO: 12 - protein, 8 aa, Artificial Sequence
  C-terminal of PDE + linker
VGRGGGGS

SEQ ID NO: 13 - protein, 5 aa, Artificial Sequence
  C-terminal sequence
  MISC_FEATURE (4)..(4): Xaa = Gly or Ala
VTVXR

SEQ ID NO: 14 - protein, 8 aa, Artificial Sequence
  C-terminal of PDE + linker
  MISC_FEATURE (4)..(4): Xaa = Gly or Ala
  MISC_FEATURE (5)..(6): cleavage site
VTVXRGGG